European Patent Specification EP 4 083 230 B1, published December 3, 2025. Title: DIRECT AMPLIFICATION AND DETECTION OF VIRAL AND BACTERIAL PATHOGENS. Applicant: QUEST DIAGNOSTICS INVESTMENTS INCORPORATED. The sequence listing filed with the application follows.

SEQUENCE LISTING (31 sequences)

SEQ ID NO: 1 - DNA, 24 bp, Artificial Sequence
  Description of Artificial Sequence: Synthetic primer
acgctcaccgtgcccagtgagcgt

SEQ ID NO: 2 - DNA, 22 bp, Artificial Sequence
  Description of Artificial Sequence: Synthetic primer
ggcattttggacaaagcgtcta

SEQ ID NO: 3 - DNA, 25 bp, Artificial Sequence
  Description of Artificial Sequence: Synthetic primer
tcttgtcacctctgactaaggggat

SEQ ID NO: 4 - DNA, 37 bp, Artificial Sequence
  Description of Artificial Sequence: Synthetic primer
  modified_base (7)..(7): Inosine
ccgcggnattgcaaaggatgtaatggaagtgccgcgg

SEQ ID NO: 5 - DNA, 22 bp, Artificial Sequence
  Description of Artificial Sequence: Synthetic primer
  modified_base (17)..(17): Inosine
gagctgaatttcccatngagct

SEQ ID NO: 6 - DNA, 21 bp, Artificial Sequence
  Description of Artificial Sequence: Synthetic primer
agctgcaaagcaacattggag

SEQ ID NO: 7 - DNA, 35 bp, Artificial Sequence
  Description of Artificial Sequence: Synthetic primer
acgcgcttcacgaaggctccacatacacagcgcgt

SEQ ID NO: 8 - DNA, 25 bp, Artificial Sequence
  Description of Artificial Sequence: Synthetic primer
ttttctaggacattgtaytgaacag

SEQ ID NO: 9 - DNA, 26 bp, Artificial Sequence
  Description of Artificial Sequence: Synthetic primer
gcaaatatggaaacatacgtgaacaa

SEQ ID NO: 10 - DNA, 31 bp, Artificial Sequence
  Description of Artificial Sequence: Synthetic primer
acgcgcttggggcgacagtcacgtcgcgcgt

SEQ ID NO: 11 - DNA, 19 bp, Artificial Sequence
  Description of Artificial Sequence: Synthetic primer
ctcgtcgacaatggcggaa

SEQ ID NO: 12 - DNA, 18 bp, Artificial Sequence
  Description of Artificial Sequence: Synthetic primer
ttcagcgaccccgttagc

SEQ ID NO: 13 - DNA, 27 bp, Artificial Sequence
  Description of Artificial Sequence: Synthetic primer
agcggcccgggtgcccggccagccgct

SEQ ID NO: 14 - DNA, 19 bp, Artificial Sequence
  Description of Artificial Sequence: Synthetic primer
gaggacgagctggcctttc

SEQ ID NO: 15 - DNA, 29 bp, Artificial Sequence
  Description of Artificial Sequence: Synthetic primer
acgcgcttccgggcgttccgcgagcgcgt

SEQ ID NO: 16 - DNA, 19 bp, Artificial Sequence
  Description of Artificial Sequence: Synthetic primer
gaggacgagctggcctttc

SEQ ID NO: 17 - DNA, 21 bp, Artificial Sequence
  Description of Artificial Sequence: Synthetic primer
ggtggtggacaggtcgtagag

SEQ ID NO: 18 - DNA, 27 bp, Artificial Sequence
  Description of Artificial Sequence: Synthetic primer
acgcggcttctgttgtttcgaccgcgt

SEQ ID NO: 19 - DNA, 20 bp, Artificial Sequence
  Description of Artificial Sequence: Synthetic primer
ccccgctttaacacattcca

SEQ ID NO: 20 - DNA, 18 bp, Artificial Sequence
  Description of Artificial Sequence: Synthetic primer
gcagttgcaaaccgggat

SEQ ID NO: 21 - DNA, 34 bp, Artificial Sequence
  Description of Artificial Sequence: Synthetic primer
aggccacacggacacccaaagtagtcggtggcct

SEQ ID NO: 22 - DNA, 19 bp, Artificial Sequence
  Description of Artificial Sequence: Synthetic primer
cccctgaatgcggctaatc

SEQ ID NO: 23 - DNA, 22 bp, Artificial Sequence
  Description of Artificial Sequence: Synthetic primer
caattgtcaccataagcagcca

SEQ ID NO: 24 - DNA, 41 bp, Artificial Sequence
  Description of Artificial Sequence: Synthetic primer
aggcagctcaccatcaataataactgaaccagttgctgcct

SEQ ID NO: 25 - DNA, 33 bp, Artificial Sequence
  Description of Artificial Sequence: Synthetic primer
ggttagatttagatgaaaagagatattatttta

SEQ ID NO: 26 - DNA, 28 bp, Artificial Sequence
  Description of Artificial Sequence: Synthetic primer
actaatcactaattgagctgtatcagga

SEQ ID NO: 27 - DNA, 122 bp, Artificial Sequence
  Description of Artificial Sequence: Synthetic polynucleotide
ggttagatttagatgaaaagagatattattttacagatgaatatattgcagcaactggttcagttattattgatggtgaggagtattattttgatcctgatacagctcaattagtgattagt

SEQ ID NO: 28 - DNA, 45 bp, Artificial Sequence
  Description of Artificial Sequence: Synthetic primer
agcggcactccaaaaatcagcagctatcaaagcaggtgtgccgct

SEQ ID NO: 29 - DNA, 25 bp, Artificial Sequence
  Description of Artificial Sequence: Synthetic primer
aagcttaatatcttctgcgcttcgt

SEQ ID NO: 30 - DNA, 22 bp, Artificial Sequence
  Description of Artificial Sequence: Synthetic primer
taacccagtatttgccgatcaa

SEQ ID NO: 31 - DNA, 127 bp, Artificial Sequence
  Description of Artificial Sequence: Synthetic polynucleotide
taacccagtatttgccgatcaaaactttgctcgtaacgaaaaagaagcaaaagatagcgctatcacatttatccaaaaatcagcagctatcaaagcaggtgcacgaagcgcagaagatattaagctt